European Patent Application EP 4 435 003 A1, published September 25, 2024. Title: CXCL12에 대한 항체 및 이를 포함하는 탈모 치료용 조성물. Applicant: 주식회사 에피바이오텍. Application KR. The sequence listing filed with the application follows.

SEQUENCE LISTING (12 sequences)

SEQ ID NO: 1 - protein, 5 aa, synthetic construct
  REGION 1..5: note = CDRH1
SYYIH

SEQ ID NO: 2 - protein, 17 aa, synthetic construct
  REGION 1..17: note = CDRH2
WIYPGNVNTKYNEKFKG

SEQ ID NO: 3 - protein, 14 aa, synthetic construct
  REGION 1..14: note = CDRH3
CWGYYYGSSYAMDY

SEQ ID NO: 4 - protein, 11 aa, synthetic construct
  REGION 1..11: note = CDRL1
RASQSIGTSIH

SEQ ID NO: 5 - protein, 7 aa, synthetic construct
  REGION 1..7: note = CDRL2
YASESIS

SEQ ID NO: 6 - protein, 10 aa, synthetic construct
  REGION 1..10: note = CDRL3
QQSNSWPTYT

SEQ ID NO: 7 - protein, 123 aa, synthetic construct
  REGION 1..123: note = VH1
QVQLVQSGAEVKKPGASVKVSCKASGYTFTSYYIHWVRQAPGQRLEWIGWIYPGNVNTKYNEKFKGRVTITADTSASTAYMELSSLRSEDTAVYYCARCWGYYYGSSYAMDYWGQGTLVTVSS

SEQ ID NO: 8 - protein, 123 aa, synthetic construct
  REGION 1..123: note = VH2
QVQLVQSGAEVKKPGASVKVSCKASGYTFTSYYIHWVRQAPGQRLEWIGWIYPGNVNTKYNEKFKGRATITADTSASTAYMELSSLRSEDTAVYFCARCWGYYYGSSYAMDYWGQGTLVTVSS

SEQ ID NO: 9 - protein, 123 aa, synthetic construct
  REGION 1..123: note = VH3
QVQLVQSGAEVKKPGASVKVSCKASGYTFTSYYIHWVRQAPGQGLEWIGWIYPGNVNTKYNEKFKGRATITADTSASTAYMELSSLRSEDTAVYFCARCWGYYYGSSYAMDYWGQGTLVTVSS

SEQ ID NO: 10 - protein, 108 aa, synthetic construct
  REGION 1..108: note = VL1
EIVLTQSPDFQSVTPKEKVTITCRASQSIGTSIHWYQQKPDQSPKLLIKYASESISGVPSRFSGSGSGTDFTLTINSLEAEDAATYYCQQSNSWPTYTFGGGTKLEIK

SEQ ID NO: 11 - protein, 108 aa, synthetic construct
  REGION 1..108: note = VL2
EIVLTQSPDFQSVTPKEKVTITCRASQSIGTSIHWYQQKPDQSPRLLIKYASESISGVPSRFSGSGSGTDFTLTINSLEAEDAADYYCQQSNSWPTYTFGGGTKLEIK

SEQ ID NO: 12 - protein, 108 aa, synthetic construct
  REGION 1..108: note = VL3
EIVLTQSPDFQSVTPKEKVTFTCRASQSIGTSIHWYQQKPDQSPRLLIKYASESISGIPSRFSGSGSGTDFTLTINSLEAEDAADYYCQQSNSWPTYTFGGGTKLEIK